European Patent Application EP 4 786 498 A1, published August 5, 2026. Title: 用于治疗肿瘤的抗PD-L1和抗4-1BB双特异性抗体. Applicant: 南京维立志博生物科技股份有限公司. Application WO. The sequence listing filed with the application follows.

SEQUENCE LISTING (48 sequences)

SEQ ID NO: 1 - protein, 5 aa, synthetic construct
SYAMH

SEQ ID NO: 2 - protein, 17 aa, synthetic construct
VISYDGSKKWYADSVKG

SEQ ID NO: 3 - protein, 15 aa, synthetic construct
NQGSGSYLYYYYMDV

SEQ ID NO: 4 - protein, 14 aa, synthetic construct
TGTSSDVGGYNYVS

SEQ ID NO: 5 - protein, 7 aa, synthetic construct
EVSNRPS

SEQ ID NO: 6 - protein, 11 aa, synthetic construct
SSYTSSSTFYV

SEQ ID NO: 7 - protein, 124 aa, synthetic construct
QVQLQESGGGLVQPGGSLRLSCAVSGFTFSSYAMHWVRQAPGKGLEWVAVISYDGSKKWYADSVKGRFTISRDNSKNTLYLQMNSLRAEDTAVYYCARNQGSGSYLYYYYMDVWGKGTTVTVSS

SEQ ID NO: 8 - protein, 112 aa, synthetic construct
  REGION 1..112: note = VARIANT 112
  SITE 112: note = Xaa can be Ser or Gly
QSALTQPRSVSGSPGQSVTISCTGTSSDVGGYNYVSWYQQLPGKAPKVIIYEVSNRPSGVSNRFSGSKSGNTASLTISGVQSEDEADYYCSSYTSSSTFYVFGTGTQLTVLX

SEQ ID NO: 9 - protein, 124 aa, synthetic construct
QVQLQESGGGLVQPGGSLRLSCAVSGFTFSSYAMHWVRQAPGKCLEWVAVISYDGSKKWYADSVKGRFTISRDNSKNTLYLQMNSLRAEDTAVYYCARNQGSGSYLYYYYMDVWGKGTTVTVSS

SEQ ID NO: 10 - protein, 111 aa, synthetic construct
QSALTQPRSVSGSPGQSVTISCTGTSSDVGGYNYVSWYQQLPGKAPKVIIYEVSNRPSGVSNRFSGSKSGNTASLTISGVQSEDEADYYCSSYTSSSTFYVFGCGTQLTVL

SEQ ID NO: 11 - protein, 5 aa, synthetic construct
SGYWN

SEQ ID NO: 12 - protein, 16 aa, synthetic construct
YVSYTGSTYYIPSLKS

SEQ ID NO: 13 - protein, 11 aa, synthetic construct
YRDWLHGYFDY

SEQ ID NO: 14 - protein, 11 aa, synthetic construct
KASQNVMDNVA

SEQ ID NO: 15 - protein, 7 aa, synthetic construct
SASYRFS

SEQ ID NO: 16 - protein, 9 aa, synthetic construct
QQYNGYPLT

SEQ ID NO: 17 - protein, 119 aa, synthetic construct
EVQLQESGPGLVKPSQTLSLTCTVSGDSFSSGYWNWIRQHPGKGLEYIGYVSYTGSTYYIPSLKSRVTISRDTSKNQFSLKLSSVTAADTAVYYCAGYRDWLHGYFDYWGQGTTVTVSS

SEQ ID NO: 18 - protein, 107 aa, synthetic construct
DIQMTQSPSSLSASVGDRVTITCKASQNVMDNVAWYQQKPGKAPKRLIYSASYRFSGVPSRFSGSGSGTEFTLTISSLQPEDFATYYCQQYNGYPLTFGQGTKLEIK

SEQ ID NO: 19 - protein, 326 aa, synthetic construct
ASTKGPSVFPLAPCSRSTSESTAALGCLVKDYFPEPVTVSWNSGALTSGVHTFPAVLQSSGLYSLSSVVTVPSSNFGTQTYTCNVDHKPSNTKVDKTVERKCCVECPPCPAPPVAGPSVFLFPPKPKDTLMISRTPEVTCVVVDVSHEDPEVQFNWYVDGVEVHNAKTKPREEQFNSTFRVVSVLTVVHQDWLNGKEYKCKVSNKGLPAPIEKTISKTKGQPREPQVYTLPPSREEMTKNQVSLTCLVKGFYPSDIAVEWESNGQPENNYKTTPPMLDSDGSFFLYSKLTVDKSRWQQGNVFSCSVMHEALHNHYTQKSLSLSPGK

SEQ ID NO: 20 - protein, 330 aa, synthetic construct
ASTKGPSVFPLAPSSKSTSGGTAALGCLVKDYFPEPVTVSWNSGALTSGVHTFPAVLQSSGLYSLSSVVTVPSSSLGTQTYICNVNHKPSNTKVDKKVEPKSCDKTHTCPPCPAPEAAGGPSVFLFPPKPKDTLMISRTPEVTCVVVAVSHEDPEVKFNWYVDGVEVHNAKTKPREEQYNSTYRVVSVLTVLHQDWLNGKEYKCKVSNKALAAPIEKTISKAKGQPREPQVYTLPPSRDELTKNQVSLTCLVKGFYPSDIAVEWESNGQPENNYKTTPPVLDSDGSFFLYSKLTVDKSRWQQGNVFSCSVMHEALHNHYTQKSLSLSPGK

SEQ ID NO: 21 - protein, 105 aa, synthetic construct
QPKAAPSVTLFPPSSEELQANKATLVCLISDFYPGAVTVAWKADSSPVKAGVETTTPSKQSNNKYAASSYLSLTPEQWKSHRSYSCQVTHEGSTVEKTVAPTECS

SEQ ID NO: 22 - protein, 107 aa, synthetic construct [sequence omitted]

SEQ ID NO: 23 - protein, 5 aa, synthetic construct
  REPEAT 1..5: note = The amino acid sequence can be repeated 1, 2, 3, 4, 5, or 6 times
GGGGS

SEQ ID NO: 24 - protein, 15 aa, synthetic construct
GSSSSGSSSSGSSSS

SEQ ID NO: 25 - protein, 714 aa, synthetic construct
EVQLQESGPGLVKPSQTLSLTCTVSGDSFSSGYWNWIRQHPGKGLEYIGYVSYTGSTYYIPSLKSRVTISRDTSKNQFSLKLSSVTAADTAVYYCAGYRDWLHGYFDYWGQGTTVTVSSASTKGPSVFPLAPSSKSTSGGTAALGCLVKDYFPEPVTVSWNSGALTSGVHTFPAVLQSSGLYSLSSVVTVPSSSLGTQTYICNVNHKPSNTKVDKKVEPKSCDKTHTCPPCPAPEAAGGPSVFLFPPKPKDTLMISRTPEVTCVVVAVSHEDPEVKFNWYVDGVEVHNAKTKPREEQYNSTYRVVSVLTVLHQDWLNGKEYKCKVSNKALAAPIEKTISKAKGQPREPQVYTLPPSRDELTKNQVSLTCLVKGFYPSDIAVEWESNGQPENNYKTTPPVLDSDGSFFLYSKLTVDKSRWQQGNVFSCSVMHEALHNHYTQKSLSLSPGKGGGGSGGGGSGGGGSQVQLQESGGGLVQPGGSLRLSCAVSGFTFSSYAMHWVRQAPGKCLEWVAVISYDGSKKWYADSVKGRFTISRDNSKNTLYLQMNSLRAEDTAVYYCARNQGSGSYLYYYYMDVWGKGTTVTVSSGSSSSGSSSSGSSSSQSALTQPRSVSGSPGQSVTISCTGTSSDVGGYNYVSWYQQLPGKAPKVIIYEVSNRPSGVSNRFSGSKSGNTASLTISGVQSEDEADYYCSSYTSSSTFYVFGCGTQLTVL

SEQ ID NO: 26 - protein, 214 aa, synthetic construct
DIQMTQSPSSLSASVGDRVTITCKASQNVMDNVAWYQQKPGKAPKRLIYSASYRFSGVPSRFSGSGSGTEFTLTISSLQPEDFATYYCQQYNGYPLTFGQGTKLEIKRTVAAPSVFIFPPSDEQLKSGTASVVCLLNNFYPREAKVQWKVDNALQSGNSQESVTEQDSKDSTYSLSSTLTLSKADYEKHKVYACEVTHQGLSSPVTKSFNRGEC

SEQ ID NO: 27 - DNA, 15 bp, synthetic construct
  source 1..15: mol_type = other DNA
agctacgccatgcac

SEQ ID NO: 28 - DNA, 42 bp, synthetic construct
  source 1..42: mol_type = other DNA
tacgacggcagcaagaagtggtatgctgatagcgtgaagggc

SEQ ID NO: 29 - DNA, 45 bp, synthetic construct
  source 1..45: mol_type = other DNA
aatcagggcagcggctcttatctgtactattactatatggacgtg

SEQ ID NO: 30 - DNA, 42 bp, synthetic construct
  source 1..42: mol_type = other DNA
acaggcacctcctccgacgtgggcggctacaactacgtgagc

SEQ ID NO: 31 - DNA, 21 bp, synthetic construct
  source 1..21: mol_type = other DNA
gaggtgtccaacaggccctcc

SEQ ID NO: 32 - DNA, 33 bp, synthetic construct
  source 1..33: mol_type = other DNA
tcctcctacacctccagctccaccttctacgtg

SEQ ID NO: 33 - DNA, 372 bp, synthetic construct
  source 1..372: mol_type = other DNA
caggtgcagctgcaggagtccggaggaggactggtgcagccaggaggctccctgaggctgagctgcgccgtgtctggcttcaccttttccagctacgccatgcactgggtgagacaggctcctggcaagtgcctggagtgggtggccgtgatctcctacgacggcagcaagaagtggtatgctgatagcgtgaagggcaggttcaccatctctcgggacaactccaagaatacactgtacctgcagatgaactctctgagagccgaggataccgccgtgtactattgtgctcgcaatcagggcagcggctcttatctgtactattactatatggacgtgtggggcaagggcaccacagtgacagtgtcttcc

SEQ ID NO: 34 - DNA, 333 bp, synthetic construct
  source 1..333: mol_type = other DNA
cagtccgccctgacccagcctaggtccgtgtccggaagccctggccagtccgtgaccatctcctgtacaggcacctcctccgacgtgggcggctacaactacgtgagctggtaccagcagctgcccggcaaggctcccaaggtgatcatctacgaggtgtccaacaggccctccggcgtgtccaataggttcagcggctccaagtccggaaacaccgcctccctgaccatcagcggcgtgcagtccgaggatgaggccgactactactgctcctcctacacctccagctccaccttctacgtgttcggctgcggcacccagctgaccgtgctg

SEQ ID NO: 35 - DNA, 15 bp, synthetic construct
  source 1..15: mol_type = other DNA
tccggctactggaac

SEQ ID NO: 36 - DNA, 48 bp, synthetic construct
  source 1..48: mol_type = other DNA
tacgtgtcctacaccggctctacctactacatccccagcctgaagtcc

SEQ ID NO: 37 - DNA, 33 bp, synthetic construct
  source 1..33: mol_type = other DNA
tacagagattggctgcacggctacttcgactac

SEQ ID NO: 38 - DNA, 33 bp, synthetic construct
  source 1..33: mol_type = other DNA
aaggccagccagaacgtgatggacaacgtggcc

SEQ ID NO: 39 - DNA, 21 bp, synthetic construct
  source 1..21: mol_type = other DNA
tccgcctcctacagattctct

SEQ ID NO: 40 - DNA, 27 bp, synthetic construct
  source 1..27: mol_type = other DNA
cagcagtacaacggctaccctctgacc

SEQ ID NO: 41 - DNA, 357 bp, synthetic construct
  source 1..357: mol_type = other DNA
gaggtccagctgcaagaatctggccctggactggtcaagccctctcagaccctgtctctgacctgtaccgtgtccggcgactccttctcttccggctactggaactggatcagacagcaccctggcaagggcctcgagtacatcggctacgtgtcctacaccggctctacctactacatccccagcctgaagtccagagtgaccatctctcgggacacctccaagaaccagttctccctgaagctgtcctccgtgaccgctgctgataccgccgtgtactactgtgccggctacagagattggctgcacggctacttcgactactggggccagggcacaacagtgaccgtttcttct

SEQ ID NO: 42 - DNA, 321 bp, synthetic construct
  source 1..321: mol_type = other DNA
gacatccagatgacccagtctccatcctctctgtccgcctctgtgggcgacagagtgaccatcacatgcaaggccagccagaacgtgatggacaacgtggcctggtatcagcagaagcctggcaaggcccctaagcggctgatctactccgcctcctacagattctctggcgtgccctctagattctccggctctggctctggcaccgagtttaccctgacaatctccagcctgcagcctgaggacttcgccacctactactgccagcagtacaacggctaccctctgacctttggccagggcaccaagctggaaatcaag

SEQ ID NO: 43 - DNA, 990 bp, synthetic construct
  source 1..990: mol_type = other DNA
gccagcaccaagggaccatccgtgttcccactggccccctccagcaagtccaccagcggaggaacagccgctctgggatgcctggtgaaggactacttcccagagcccgtgacagtgagctggaactctggcgccctgaccagcggagtgcacacatttcccgccgtgctccagtcttccggcctgtactctctgagctctgtggtgaccgtgccctccagctctctgggcacccagacatatatctgcaacgtgaatcacaagccaagcaatacaaaggtggacaagaaggtggagcccaagtcttgtgataagacccatacatgccccccttgtcctgctccagaggctgctggaggaccaagcgtgttcctgtttccacccaagcctaaggacaccctgatgatctccaggacccccgaggtgacatgcgtggtggtggctgtgagccacgaggaccccgaggtgaagtttaactggtacgtggatggcgtggaggtgcataatgctaagaccaagcctagggaggagcagtacaactctacctatcgggtggtgtccgtgctgacagtgctgcaccaggactggctgaacggcaaggagtataagtgcaaggtgtctaataaggccctggctgctcctatcgagaagaccatctccaaggccaagggccagcctagagagccacaggtgtacacactgcctccatctcgcgacgagctgaccaagaaccaggtgtccctgacatgtctggtgaagggcttctatccttccgacatcgctgtggagtgggagagcaacggccagccagagaacaattacaagaccacaccccctgtgctggactccgatggcagcttctttctgtatagcaagctgaccgtggataagtccaggtggcagcagggcaacgtgttttcttgctccgtgatgcatgaggctctgcacaatcattatacacagaagagcctgtctctgtcccctggcaag

SEQ ID NO: 44 - DNA, 321 bp, synthetic construct
  source 1..321: mol_type = other DNA
cggacggtggctgcaccatctgtcttcatcttcccgccatctgatgagcagttgaaatctggaactgcctctgttgtgtgcctgctgaataacttctaccccagagaagccaaagtgcagtggaaggtggacaacgccctgcagagcggaaacagccaggaaagcgtgacagagcaggattccaaggattccacatacagcctgagcagcacactgacactgtccaaggccgactacgagaagcacaaggtgtacgcctgcgaagtgacacaccagggactgtcctcccctgtgacaaagagcttcaacagaggagaatgc

SEQ ID NO: 45 - DNA, 2142 bp, synthetic construct
  source 1..2142: mol_type = other DNA
gaggtccagctgcaagaatctggccctggactggtcaagccctctcagaccctgtctctgacctgtaccgtgtccggcgactccttctcttccggctactggaactggatcagacagcaccctggcaagggcctcgagtacatcggctacgtgtcctacaccggctctacctactacatccccagcctgaagtccagagtgaccatctctcgggacacctccaagaaccagttctccctgaagctgtcctccgtgaccgctgctgataccgccgtgtactactgtgccggctacagagattggctgcacggctacttcgactactggggccagggcacaacagtgaccgtttcttctgccagcaccaagggaccatccgtgttcccactggccccctccagcaagtccaccagcggaggaacagccgctctgggatgcctggtgaaggactacttcccagagcccgtgacagtgagctggaactctggcgccctgaccagcggagtgcacacatttcccgccgtgctccagtcttccggcctgtactctctgagctctgtggtgaccgtgccctccagctctctgggcacccagacatatatctgcaacgtgaatcacaagccaagcaatacaaaggtggacaagaaggtggagcccaagtcttgtgataagacccatacatgccccccttgtcctgctccagaggctgctggaggaccaagcgtgttcctgtttccacccaagcctaaggacaccctgatgatctccaggacccccgaggtgacatgcgtggtggtggctgtgagccacgaggaccccgaggtgaagtttaactggtacgtggatggcgtggaggtgcataatgctaagaccaagcctagggaggagcagtacaactctacctatcgggtggtgtccgtgctgacagtgctgcaccaggactggctgaacggcaaggagtataagtgcaaggtgtctaataaggccctggctgctcctatcgagaagaccatctccaaggccaagggccagcctagagagccacaggtgtacacactgcctccatctcgcgacgagctgaccaagaaccaggtgtccctgacatgtctggtgaagggcttctatccttccgacatcgctgtggagtgggagagcaacggccagccagagaacaattacaagaccacaccccctgtgctggactccgatggcagcttctttctgtatagcaagctgaccgtggataagtccaggtggcagcagggcaacgtgttttcttgctccgtgatgcatgaggctctgcacaatcattatacacagaagagcctgtctctgtcccctggcaagggtggcggaggatctggcggaggcggaagtggcggtggcggttcacaggtgcagctgcaggagtccggaggaggactggtgcagccaggaggctccctgaggctgagctgcgccgtgtctggcttcaccttttccagctacgccatgcactgggtgagacaggctcctggcaagtgcctggagtgggtggccgtgatctcctacgacggcagcaagaagtggtatgctgatagcgtgaagggcaggttcaccatctctcgggacaactccaagaatacactgtacctgcagatgaactctctgagagccgaggataccgccgtgtactattgtgctcgcaatcagggcagcggctcttatctgtactattactatatggacgtgtggggcaagggcaccacagtgacagtgtcttccggctcctccagctctggcagttctagctctggctctagctccagccagtccgccctgacccagcctaggtccgtgtccggaagccctggccagtccgtgaccatctcctgtacaggcacctcctccgacgtgggcggctacaactacgtgagctggtaccagcagctgcccggcaaggctcccaaggtgatcatctacgaggtgtccaacaggccctccggcgtgtccaataggttcagcggctccaagtccggaaacaccgcctccctgaccatcagcggcgtgcagtccgaggatgaggccgactactactgctcctcctacacctccagctccaccttctacgtgttcggctgcggcacccagctgaccgtgctg

SEQ ID NO: 46 - DNA, 642 bp, synthetic construct
  source 1..642: mol_type = other DNA
gacatccagatgacccagtctccatcctctctgtccgcctctgtgggcgacagagtgaccatcacatgcaaggccagccagaacgtgatggacaacgtggcctggtatcagcagaagcctggcaaggcccctaagcggctgatctactccgcctcctacagattctctggcgtgccctctagattctccggctctggctctggcaccgagtttaccctgacaatctccagcctgcagcctgaggacttcgccacctactactgccagcagtacaacggctaccctctgacctttggccagggcaccaagctggaaatcaagcggacggtggctgcaccatctgtcttcatcttcccgccatctgatgagcagttgaaatctggaactgcctctgttgtgtgcctgctgaataacttctaccccagagaagccaaagtgcagtggaaggtggacaacgccctgcagagcggaaacagccaggaaagcgtgacagagcaggattccaaggattccacatacagcctgagcagcacactgacactgtccaaggccgactacgagaagcacaaggtgtacgcctgcgaagtgacacaccagggactgtcctcccctgtgacaaagagcttcaacagaggagaatgc

SEQ ID NO: 47 - protein, 15 aa, synthetic construct
GGGGSGGGGSGGGGS

SEQ ID NO: 48 - protein, 255 aa, synthetic construct
MGNSCYNIVATLLLVLNFERTRSLQDPCSNCPAGTFCDNNRNQICSPCPPNSFSSAGGQRTCDICRQCKGVFRTRKECSSTSNAECDCTPGFHCLGAGCSMCEQDCKQGQELTKKGCKDCCFGTFNDQKRGICRPWTNCSLDGKSVLVNGTKERDVVCGPSPADLSPGASSVTPPAPAREPGHSPQIISFFLALTSTALLFLLFFLTLRFSVVKRGRKKLLYIFKQPFMRPVQTTQEEDGCSCRFPEEEEGGCEL